European Patent Application EP 4 759 832 A1, published June 17, 2026. Title: ANTIGEN-BINDING POLYPEPTIDES AGAINST CD203a. Applicant: Universitätsklinikum Hamburg-Eppendorf. The sequence listing filed with the application follows.

SEQUENCE LISTING (173 sequences)

SEQ ID NO: 1 - protein, 6 aa, Vicugna pacos
TFDDYA

SEQ ID NO: 2 - protein, 6 aa, Vicugna pacos
SANDGT

SEQ ID NO: 3 - protein, 16 aa, Vicugna pacos
EVRECRTRDEYWLYDL

SEQ ID NO: 4 - protein, 6 aa, Vicugna pacos
TFDDYA

SEQ ID NO: 5 - protein, 6 aa, Vicugna pacos
SANDGT

SEQ ID NO: 6 - protein, 17 aa, Vicugna pacos
EVREWCRTRDEFWLYDL

SEQ ID NO: 7 - protein, 6 aa, Vicugna pacos
TLANYA

SEQ ID NO: 8 - protein, 5 aa, Vicugna pacos
RYDGS

SEQ ID NO: 9 - protein, 14 aa, Vicugna pacos
VSPRYGSPDCAYDF

SEQ ID NO: 10 - protein, 6 aa, Vicugna pacos
TFSSGF

SEQ ID NO: 11 - protein, 6 aa, Vicugna pacos
GWNSGN

SEQ ID NO: 12 - protein, 17 aa, Vicugna pacos
TAPDFGGRVSGEATYQY

SEQ ID NO: 13 - protein, 6 aa, Vicugna pacos
TFSSGF

SEQ ID NO: 14 - protein, 6 aa, Vicugna pacos
GWNSGN

SEQ ID NO: 15 - protein, 17 aa, Vicugna pacos
TAPDFGGSVSKEVTYQY

SEQ ID NO: 16 - protein, 6 aa, Vicugna pacos
TFSSGF

SEQ ID NO: 17 - protein, 6 aa, Vicugna pacos
GWNSGN

SEQ ID NO: 18 - protein, 17 aa, Vicugna pacos
TAPDFGGSVSNEATYQY

SEQ ID NO: 19 - protein, 6 aa, Vicugna pacos
TFSTGF

SEQ ID NO: 20 - protein, 6 aa, Vicugna pacos
GWNSGN

SEQ ID NO: 21 - protein, 17 aa, Vicugna pacos
TAPDFGGRVSNEATYQY

SEQ ID NO: 22 - protein, 6 aa, Vicugna pacos
TNRHYL

SEQ ID NO: 23 - protein, 6 aa, Vicugna pacos
NWRADS

SEQ ID NO: 24 - protein, 20 aa, Vicugna pacos
EWTWVDGSKATMLGRSTADY

SEQ ID NO: 25 - protein, 6 aa, Vicugna pacos
TLDPYA

SEQ ID NO: 26 - protein, 6 aa, Vicugna pacos
RRRDYN

SEQ ID NO: 27 - protein, 19 aa, Vicugna pacos
APDYSGIYCLTSSYRYLDL

SEQ ID NO: 28 - protein, 6 aa, Vicugna pacos
TLDHYA

SEQ ID NO: 29 - protein, 6 aa, Vicugna pacos
RRRDYN

SEQ ID NO: 30 - protein, 19 aa, Vicugna pacos
APEYSGIYCLTSSYRYLDL

SEQ ID NO: 31 - protein, 6 aa, Vicugna pacos
FFAING

SEQ ID NO: 32 - protein, 5 aa, Vicugna pacos
TSKGS

SEQ ID NO: 33 - protein, 13 aa, Vicugna pacos
EVVSNLHYYGMDY

SEQ ID NO: 34 - protein, 6 aa, Vicugna pacos
TFSINT

SEQ ID NO: 35 - protein, 8 aa, Vicugna pacos
AEISSGGS

SEQ ID NO: 36 - protein, 15 aa, Vicugna pacos
DGDYSDYGRYYGREY

SEQ ID NO: 37 - protein, 6 aa, Vicugna pacos
TFSINT

SEQ ID NO: 38 - protein, 8 aa, Vicugna pacos
AEISSGGS

SEQ ID NO: 39 - protein, 15 aa, Vicugna pacos
DGDYSDYGRYYGREY

SEQ ID NO: 40 - protein, 6 aa, Vicugna pacos
TFSIDT

SEQ ID NO: 41 - protein, 8 aa, Vicugna pacos
AEISRGGS

SEQ ID NO: 42 - protein, 15 aa, Vicugna pacos
IGDYSDYGRYYGRDY

SEQ ID NO: 43 - protein, 6 aa, Vicugna pacos
TFSSDA

SEQ ID NO: 44 - protein, 6 aa, Vicugna pacos
NRSGAI

SEQ ID NO: 45 - protein, 15 aa, Vicugna pacos
RTTVVHTTDTTSYNS

SEQ ID NO: 46 - protein, 6 aa, Vicugna pacos
TFGRDA

SEQ ID NO: 47 - protein, 6 aa, Vicugna pacos
AKSGAP

SEQ ID NO: 48 - protein, 15 aa, Vicugna pacos
RTTVVHTADTTSYDS

SEQ ID NO: 49 - protein, 6 aa, Vicugna pacos
SLEDYT

SEQ ID NO: 50 - protein, 6 aa, Vicugna pacos
RSNDDN

SEQ ID NO: 51 - protein, 26 aa, Vicugna pacos
DRVFEKCVAIASLPTAPPRNGGYLEV

SEQ ID NO: 52 - protein, 8 aa, Vicugna pacos
SLDLKYYA

SEQ ID NO: 53 - protein, 8 aa, Vicugna pacos
TSSVTQGR

SEQ ID NO: 54 - protein, 19 aa, Vicugna pacos
ADSGYGCYSHRSSSYDYEH

SEQ ID NO: 55 - protein, 6 aa, Vicugna pacos
TFTAYA

SEQ ID NO: 56 - protein, 6 aa, Vicugna pacos
SWNGAI

SEQ ID NO: 57 - protein, 20 aa, Vicugna pacos
AQTVPVRGSWYDITPGAYDY

SEQ ID NO: 58 - protein, 6 aa, Vicugna pacos
TFTAYA

SEQ ID NO: 59 - protein, 6 aa, Vicugna pacos
SWNGAI

SEQ ID NO: 60 - protein, 20 aa, Vicugna pacos
AQTVPVRGSWYDITPGAYDY

SEQ ID NO: 61 - protein, 6 aa, Vicugna pacos
LDNYAI

SEQ ID NO: 62 - protein, 5 aa, Vicugna pacos
TNAYS

SEQ ID NO: 63 - protein, 19 aa, Vicugna pacos
VPLYGHYYCTGPGRAGMDH

SEQ ID NO: 64 - protein, 6 aa, Vicugna pacos
THGDFG

SEQ ID NO: 65 - protein, 5 aa, Vicugna pacos
YSRDT

SEQ ID NO: 66 - protein, 19 aa, Vicugna pacos
TEYQIYNAYVCPKGRGMDF

SEQ ID NO: 67 - protein, 6 aa, Vicugna pacos
RFDDHS

SEQ ID NO: 68 - protein, 6 aa, Vicugna pacos
SFRDGR

SEQ ID NO: 69 - protein, 18 aa, Vicugna pacos
RDYYSCPTDRPPFMTSGY

SEQ ID NO: 70 - protein, 6 aa, Vicugna pacos
SLGDYA

SEQ ID NO: 71 - protein, 8 aa, Vicugna pacos
TSNDVISR

SEQ ID NO: 72 - protein, 18 aa, Vicugna pacos
MPDMFCSTSGLRNNPVHS

SEQ ID NO: 73 - protein, 6 aa, Vicugna pacos
TSSSLA

SEQ ID NO: 74 - protein, 6 aa, Vicugna pacos
NWSGSS

SEQ ID NO: 75 - protein, 17 aa, Vicugna pacos
DYASPVDWHLGGAGYDF

SEQ ID NO: 76 - protein, 6 aa, Vicugna pacos
TFGTYT

SEQ ID NO: 77 - protein, 6 aa, Vicugna pacos
SWSGGS

SEQ ID NO: 78 - protein, 17 aa, Vicugna pacos
QERNRYTDSREADDYRS

SEQ ID NO: 79 - protein, 6 aa, Vicugna pacos
INAIDT

SEQ ID NO: 80 - protein, 5 aa, Vicugna pacos
SDLNI

SEQ ID NO: 81 - protein, 14 aa, Vicugna pacos
NIQQYPTLAPRRIL

SEQ ID NO: 82 - protein, 6 aa, Vicugna pacos
TDSIYG

SEQ ID NO: 83 - protein, 5 aa, Vicugna pacos
RNDGN

SEQ ID NO: 84 - protein, 12 aa, Vicugna pacos
GYLYGLGPEYDY

SEQ ID NO: 85 - protein, 6 aa, Vicugna pacos
IFGDVT

SEQ ID NO: 86 - protein, 5 aa, Vicugna pacos
KSDGS

SEQ ID NO: 87 - protein, 12 aa, Vicugna pacos
ESREWGLPPVHY

SEQ ID NO: 88 - protein, 6 aa, Vicugna pacos
TDSING

SEQ ID NO: 89 - protein, 5 aa, Vicugna pacos
STGGS

SEQ ID NO: 90 - protein, 9 aa, Vicugna pacos
RRLPWGADY

SEQ ID NO: 91 - protein, 6 aa, Vicugna pacos
TDSINA

SEQ ID NO: 92 - protein, 5 aa, Vicugna pacos
STGGS

SEQ ID NO: 93 - protein, 9 aa, Vicugna pacos
RRLPWGADY

SEQ ID NO: 94 - protein, 6 aa, Vicugna pacos
NFNNIA

SEQ ID NO: 95 - protein, 6 aa, Vicugna pacos
SSGSST

SEQ ID NO: 96 - protein, 6 aa, Vicugna pacos
MAPYQP

SEQ ID NO: 97 - protein, 6 aa, Vicugna pacos
LSIDVM

SEQ ID NO: 98 - protein, 4 aa, Vicugna pacos
  source 1..4: note = only amino acids 1-3 (R-G-K) represent the CDR, while the amino acid T does not belong to the CDR
RGKT

SEQ ID NO: 99 - protein, 5 aa, Vicugna pacos
GWGDY

SEQ ID NO: 100 - protein, 6 aa, Vicugna pacos
PFSTFT

SEQ ID NO: 101 - protein, 6 aa, Vicugna pacos
NGGGGT

SEQ ID NO: 102 - protein, 5 aa, Vicugna pacos
QSQRP

SEQ ID NO: 103 - protein, 6 aa, Vicugna pacos
TFSGNF

SEQ ID NO: 104 - protein, 5 aa, Vicugna pacos
SRSGK

SEQ ID NO: 105 - protein, 4 aa, Vicugna pacos
SPGD

SEQ ID NO: 106 - protein, 6 aa, Vicugna pacos
IASIYA

SEQ ID NO: 107 - protein, 5 aa, Vicugna pacos
TTDGV

SEQ ID NO: 108 - protein, 23 aa, Vicugna pacos
VPMRGPGVDGIGVDISMTTLVGY

SEQ ID NO: 109 - protein, 6 aa, Vicugna pacos
TFSIDT

SEQ ID NO: 110 - protein, 4 aa, Vicugna pacos
SGGS

SEQ ID NO: 111 - protein, 15 aa, Vicugna pacos
NGDYSDYGRYYGREY

SEQ ID NO: 112 - protein, 6 aa, Vicugna pacos
TFGINA

SEQ ID NO: 113 - protein, 5 aa, Vicugna pacos
SSGGN

SEQ ID NO: 114 - protein, 15 aa, Vicugna pacos
NGDYSDYGRYYGREY

SEQ ID NO: 115 - protein, 6 aa, Vicugna pacos
DFAYYG

SEQ ID NO: 116 - protein, 7 aa, Vicugna pacos
TSGGSTD

SEQ ID NO: 117 - protein, 11 aa, Vicugna pacos
RRGGYGTGPEY

SEQ ID NO: 118 - protein, 6 aa, Vicugna pacos
KIGIYT

SEQ ID NO: 119 - protein, 5 aa, Vicugna pacos
TSGEH

SEQ ID NO: 120 - protein, 7 aa, Vicugna pacos
RSITFDF

SEQ ID NO: 121 - protein, 6 aa, Vicugna pacos
TFSNSW

SEQ ID NO: 122 - protein, 6 aa, Vicugna pacos
RGDGGE

SEQ ID NO: 123 - protein, 5 aa, Vicugna pacos
AGWGY

SEQ ID NO: 124 - protein, 6 aa, Vicugna pacos
TANRYA

SEQ ID NO: 125 - protein, 4 aa, Vicugna pacos
DDGL

SEQ ID NO: 126 - protein, 17 aa, Vicugna pacos
RYTSFTDSWSDWSDYDS

SEQ ID NO: 127 - protein, 6 aa, Vicugna pacos
TSRIRT

SEQ ID NO: 128 - protein, 5 aa, Vicugna pacos
SRGGS

SEQ ID NO: 129 - protein, 15 aa, Vicugna pacos
NGDYSDYGRYYGREY

SEQ ID NO: 130 - protein, 127 aa, Vicugna pacos
MSQVQLVESGGGLVQAGGSLRLSCAASGFTFDDYAIGWFRQAPGKEREGVSCISANDGTTYYRDSVQGRFTISSDNAKNTVYLQMNSLKPEDTAVYYCAAEVRECRTRDEYWLYDLTGQGTQVTVSS

SEQ ID NO: 131 - protein, 128 aa, Vicugna pacos
MSQVQLVESGGGLVQAGGSLRLSCAASGFTFDDYAIGWFRQAPGKEREGVSCISANDGTTYYVDSVQGRFTISSDNAKNTVYLQMNSLKPEDTAVYYCAAEVREWCRTRDEFWLYDLTGQGTQVTVSS

SEQ ID NO: 132 - protein, 124 aa, Vicugna pacos
MSQVQLVESGGGLVQPGGSLRLSCAASGITLANYAMGWFRQAPGKEREGVSCIRYDGSTIYADSVRGRFTFSRDNAKNMVYLQMNSLKPEDTAVYYCATVSPRYGSPDCAYDFWGQGTQITVSS

SEQ ID NO: 133 - protein, 128 aa, Vicugna pacos
MSQVQLVESGGGLVQAGDSLRLSCTTSGRTFSSGFMGWFRQAPGKEREFVAGFGWNSGNRYYAESVKGRFTISRDNAKNAVYLQMNSLKPEDTGVYYCASTAPDFGGRVSGEATYQYWGQGTQVTVSS

SEQ ID NO: 134 - protein, 128 aa, Vicugna pacos
MSQVQLVESGGGLVQAGDSLRLSCTTSGRTFSSGFMGWFRQAPGKEREFVAGFGWNSGNRYYAESVKGRFTISRDNAKNAVYLQMNSLKPEDTGVYYCASTAPDFGGSVSKEVTYQYWGQGTQVTVSS

SEQ ID NO: 135 - protein, 128 aa, Vicugna pacos
MSQVQLVESGGGLVQAGDSLRLSCTTSGRTFSSGFMGWFRQAPGKEREFVAGFGWNSGNRYYAESVKGRFTISRDNAKNAVYLQMNSLKPEDTGVYYCASTAPDFGGSVSNEATYQYWGQGTQVTVSS

SEQ ID NO: 136 - protein, 128 aa, Vicugna pacos
MSQVQLVESGGGLVQAGDSLRLSCTTSGRTFSTGFMGWFRQAPGKEREFVAGFGWNSGNRYYAESVKGRFTISRDNAKNAVYLQMNNLKPEDTGVYYCASTAPDFGGRVSNEATYQYWGQGTQVTVSS

SEQ ID NO: 137 - protein, 131 aa, Vicugna pacos
MSQVQLVESGGGLVQAGGSLRLSCTFSNPTNRHYLLGWFRQAPGKEREFLASVNWRADSTFYANSVKGRFTISRDNAKNTMYLQMNSLRPEDTAVYYCAAEWTWVDGSKATMLGRSTADYWGKGTLVTVSS

SEQ ID NO: 138 - protein, 130 aa, Vicugna pacos
MSQVQLVESGGGLVQTGGSLRLSCRVSGFTLDPYAIGWFRQAPGKEREGVSCIRRRDYNTYYADSVKGRFTASIDNAKNTVYLQMNSLQPEDTAVYYCARAPDYSGIYCLTSSYRYLDLWGQGTLVTVSS

SEQ ID NO: 139 - protein, 130 aa, Vicugna pacos
MSQVQLVESGGDSVQTGGSLRLSCAVSGFTLDHYAIGWFRQAPGKEREGVSCIRRRDYNTYYVDSVKGRFTASIDNAKNTVYLQMNDLQPEDTAVYYCARAPEYSGIYCLTSSYRYLDLWGQGTLVTVSS

SEQ ID NO: 140 - protein, 123 aa, Vicugna pacos
MSQVQLVESGGALVQPGGSLRLSCAASGIFFAINGMGWYRQAPGKQRELVAEITSKGSTNYADSVNGRFTISRDNGKNTVYLQMNSLKAEDTAVYYCTAEVVSNLHYYGMDYWGNGTLVTVSS

SEQ ID NO: 141 - protein, 128 aa, Vicugna pacos
MSQVQLVESGGGLVQAGGSLRLSCAASGSTFSINTMGWHRQAPGKEREERELVAEISSGGSANYADSVKGRFTISRDNAKNTVYLQMNNLKPEDTAVYYCNADGDYSDYGRYYGREYWGKGTLVTVSS

SEQ ID NO: 142 - protein, 128 aa, Vicugna pacos
MSQVQLVESGGGLVQAGGSLRLSCAASGSTFSINTMGWHRQAPGKEREEGELVAEISSGGSANYADSVKGRFTISRDNAKNTVYLQMNNLKPEDTAVYYCNADGDYSDYGRYYGREYWGKGTLVTVSS

SEQ ID NO: 143 - protein, 128 aa, Vicugna pacos
MSQVQLVESGGGLVQAGGSLRLSCAASGSTFSIDTMGWHRQAPGKEREERELVAEISRGGSANYADSVKGRFTISRDNAKNTVYLQMNNLKPEDTAVYYCNAIGDYSDYGRYYGRDYWGKGTLVTVSS

SEQ ID NO: 144 - protein, 126 aa, Vicugna pacos
MSQVQLVESGGGLVQAGGSLRLSCTASGRTFSSDAMGWFRQTPGKEREFVTAINRSGAITYYADSVKGRFTISRDNAKNTVYLQMNSLKPEDTARYYCAVRTTVVHTTDTTSYNSWGQGTQVTVSS

SEQ ID NO: 145 - protein, 126 aa, Vicugna pacos
MSQVQLVESGGGLVQAGGSLRLSCTASGSTFGRDAVGWFRQTPGKEREFVAGIAKSGAPTYYADSVKGRFTISRDNAKNTVYLQMNSLKPEDTARYYCAVRTTVVHTADTTSYDSWGQGTQVTVSS

SEQ ID NO: 146 - protein, 137 aa, Vicugna pacos
MSQVQLVESGGGLVQVGGSLKLSCIASGFSLEDYTMGWFRQVPGKDPEGLACFRSNDDNPYLAPFVKGRFTGSTNNAKNTMYLQMNNLQPEDAALYYCAADRVFEKCVAIASLPTAPPRNGGYLEVRGQGTLVTVSS

SEQ ID NO: 147 - protein, 134 aa, Vicugna pacos
MSQVQLVESGGGLAQPGGSLTLSCVVSGLSLDLKYYALGWFRQAPGKAREAVSCVTSSVTQGRTWYGDSVKGRFTISRDDAKNTMYLQMNSLKPEDTAKYYCAEADSGYGCYSHRSSSYDYEHWGQGIQVTVSS

SEQ ID NO: 148 - protein, 131 aa, Vicugna pacos
MSQVQLVESGGGLVQAGASLNLSCAASGGTFTAYAISWFRQAPGKEREYVAACSWNGAITHYSDSAKGRFNISRDNAKNMVYLHMDSLKSEDTAVYYCAAAQTVPVRGSWYDITPGAYDYWGPGTQVTVSS

SEQ ID NO: 149 - protein, 131 aa, Vicugna pacos; identical to SEQ ID NO: 148

SEQ ID NO: 150 - protein, 128 aa, Vicugna pacos
MSQVQLVESGGGLVQPGGSTRLSCTASSTLDNYAIGWFRQTPGKEREGVSCISTNAYSTIYSDSVKGRFTISRNNLDNTVSLQMNSLKPEDTGVYYCATVPLYGHYYCTGPGRAGMDHWGKGTLVNVS

SEQ ID NO: 151 - protein, 129 aa, Vicugna pacos
MSQVQLVESGGGLVQAGSSLTLSCAVSGFTHGDFGIGWFRQAPGKEREGVICFYSRDTTYYADSVEGRFTFSNDRDKNVVYLHMNNLKPEDTAVYYCAATEYQIYNAYVCPKGRGMDFWGRGTPVNVSS

SEQ ID NO: 152 - protein, 129 aa, Vicugna pacos
MSQVQLVESGGGLVQAGGSLKLSCEVSGFRFDDHSIGWFRQAPGKEREGISCFSFRDGRTYLANSVKGRFSISTDNAKKMVYLQMTNLKPEDTAVYYCAARDYYSCPTDRPPFMTSGYWGQGTQVTVSS

SEQ ID NO: 153 - protein, 131 aa, Vicugna pacos
MSQVQLVESGGGSVQPGESLRLSCGGSGFSLGDYAIGWFRQAPQKEREGISCVTSNDVISRTAYADWVQGRFIVSRDNAQNLVYLQMNMLKPEDTAVYYCATMPDMFCSTSGLRNNPVHSWGQRTQVTVFT

SEQ ID NO: 154 - protein, 128 aa, Vicugna pacos
MSQVQLVESGGGLVQAGGSLKLSCSASGRTSSSLAMAWFRQTPGKEREFVAAINWSGSSTYYGDSVKGRFTISSDNAKRTSYLQMNMLKPEDTAVYYCAADYASPVDWHLGGAGYDFWGQGTQVTVSS

SEQ ID NO: 155 - protein, 128 aa, Vicugna pacos
MSQVQLVESGGKLVRTGEPLRLSCAASRGTFGTYTVGWFRQTPGKERTFVAAISWSGGSTYYAESVLGRFILSRDNVKNTVSLQMNNLDPEDTGVYVCALQERNRYTDSREADDYRSWGQGTQVIVSS

SEQ ID NO: 156 - protein, 124 aa, Vicugna pacos
MSQVQLVESGGGLVQSGGSLRLSCVASGYINAIDTMAWYRQAPGKQREFVASISDLNIKRYSDSVKGRFSVSLESAKNTMYLQMNALQPEDTAVYYCHGNIQQYPTLAPRRILAARAIQVTVSA

SEQ ID NO: 157 - protein, 122 aa, Vicugna pacos
MSQVQLVESGGGLVQAGGSLRLSCAASGSTDSIYGMAWYRQAPGKQRELVARIRNDGNTNYADFVKGRFAISRDNAQNTLYLQMNSLKPEDTAVYYCNAGYLYGLGPEYDYWGQGTQVTVSS

SEQ ID NO: 158 - protein, 122 aa, Vicugna pacos
MSQVQLVESEGGLVQPGGSLRISCAASGSIFGDVTMAWFREGARKSRELVAVIKSDGSTNYADFVQGRFRISRDGAKYTVYLQMDSLKSEDTAVYYCDVESREWGLPPVHYWGQGIQVTVSS

SEQ ID NO: 159 - protein, 119 aa, Vicugna pacos
MSQVQLVESGGGLVQAGGSLRLSCAASGSTDSINGMGWYRQAPGKQREVVASISTGGSINYVDSVKGRFTISRDNAKNTVYLQMNSLKPDDTAVYYCNARRLPWGADYWGQGTQVTVSS

SEQ ID NO: 160 - protein, 119 aa, Vicugna pacos; identical to SEQ ID NO: 159

SEQ ID NO: 161 - protein, 119 aa, Vicugna pacos
MSQVQLVESGGGLVQAGGSLRLSCAASGSTDSINAMGWYRQAPGKQREVVAAISTGGSINYRDSVKGRFTISRDAAKNTVYLQMNSLKPDDTAVYYCNARRLPWGADYWGQGTQVTVSS

SEQ ID NO: 162 - protein, 117 aa, Vicugna pacos
MSQVQLVESGGALVQTGESLTLSCLTSLSNFNNIAMAWYRQGPGRQRETVAIISSGSSTTNYAPSVKDRFTVSRDNGKKALYLQMNELKPEDTAVYYCNSMAPYQPWGRGTQVTVSS

SEQ ID NO: 163 - protein, 113 aa, Vicugna pacos
MSQVQLVESGGGLVQAGGSLRLSCTASETLSIDVMAWYRQAPGKQREWVATIERGKTKYAESVKGRFTISGDNAKNTVYLQMNSLKPEDTAVYHCNPGWGDYWGQGTQVTVSS

SEQ ID NO: 164 - protein, 116 aa, Vicugna pacos
MSQVQLVESGGGLVQPGGSLNLSCAASGFPFSTFTMTWVRQPPGKRMEWVSSINGGGGTGIYADSVKGRFTISRDNAKNTLYLQMSDLQPEDTAIYYCTKQSQRPPGQGTQVTVSL

SEQ ID NO: 165 - protein, 114 aa, Vicugna pacos
MSQVQLVESGGGLVEAGESLRLSCAASGSTFSGNFMAWYRQAPGEQREMVAGFSRSGKELYADSVKGRFTISRDNNKNIVYLQMDNLEPEDTAVYYCYMSPGDWGQGIPVTVSS

SEQ ID NO: 166 - protein, 133 aa, Vicugna pacos
MSQVQLVESGGGLVQPGGSLRLSCLASGSIASIYAMAWYRQPPGKQRELVASITTDGVTNYADSMKGRFIISRDDTKNTVYLQMNSLRPEDTAVYCCNAVPMRGPGVDGIGVDISMTTLVGYWGQGTQVTVSS

SEQ ID NO: 167 - protein, 125 aa, Vicugna pacos
MSQVQLVESGGGLVQAGGSLRLSCAASGMTFSIDTMGWYRQAPGKQRELVASISSGGSTNYEDSVKGRFTISRDNAKNTAYLQMNSLKPEDTAVYYCNANGDYSDYGRYYGREYWGKGTLVTVSS

SEQ ID NO: 168 - protein, 125 aa, Vicugna pacos
MSQVQLVESGGGLVQAGGSLRLSCAASGSTFGINAMGWYRQAPGKQRELVAFISSGGNTNYADSVKGRFTISRVHANNTVYLQMNSLKPEDTAVYYCNANGDYSDYGRYYGREYWGKGTLVTVSS

SEQ ID NO: 169 - protein, 123 aa, Vicugna pacos
MSQVQLVESGGGAAQPGGSLKLSCVASGSDFAYYGMGWFRQTPQKQREMVATITSGGSTDYGDSVRGRFAISKDSAENTVTVYLEMNNLKPEDTAVYYCNARRGGYGTGPEYWGQGTQVTVSS

SEQ ID NO: 170 - protein, 117 aa, Vicugna pacos
MSQVQLVESGGGLVSPGGSLRLSCTASGIKIGIYTMGWYRQAPGKLREVVATSTSGEHSNYEDSVNDRFTISRDNAKNTVYLQMNTLKPEDTAVYYCNARSITFDFWGQGTQVTVSS

SEQ ID NO: 171 - protein, 116 aa, Vicugna pacos
MSQVQLVESGGGLVQPGGSLRLSCSASGFTFSNSWMYWVRQAPGKGLEWVSNIRGDGGEINYADSVKDRFTASRDNANNTMYLQLNTLKPEDTALYYCLTAGWGYWGQGTQVTVSS

SEQ ID NO: 172 - protein, 126 aa, Vicugna pacos
MSQVQLVESGGGLVQAGGSLRLSCTASGRTANRYAMAWFRQGPGKDREFVATIDDGLTYYADSVKGRFTISKDNAKNTLYLQMDRVNPEDTAVYRCALRYTSFTDSWSDWSDYDSWGQGTQVTVSS

SEQ ID NO: 173 - protein, 925 aa, Homo sapiens
MERDGCAGGGSRGGEGGRAPREGPAGNGRDRGRSHAAEAPGDPQAAASLLAPMDVGEEPLEKAARARTAKDPNTYKVLSLVLSVCVLTTILGCIFGLKPSCAKEVKSCKGRCFERTFGNCRCDAACVELGNCCLDYQETCIEPEHIWTCNKFRCGEKRLTRSLCACSDDCKDKGDCCINYSSVCQGEKSWVEEPCESINEPQCPAGFETPPTLLFSLDGFRAEYLHTWGGLLPVISKLKKCGTYTKNMRPVYPTKTFPNHYSIVTGLYPESHGIIDNKMYDPKMNASFSLKSKEKFNPEWYKGEPIWVTAKYQGLKSGTFFWPGSDVEINGIFPDIYKMYNGSVPFEERILAVLQWLQLPKDERPHFYTLYLEEPDSSGHSYGPVSSEVIKALQRVDGMVGMLMDGLKELNLHRCLNLILISDHGMEQGSCKKYIYLNKYLGDVKNIKVIYGPAARLRPSDVPDKYYSFNYEGIARNLSCREPNQHFKPYLKHFLPKRLHFAKSDRIEPLTFYLDPQWQLALNPSERKYCGSGFHGSDNVFSNMQALFVGYGPGFKHGIEADTFENIEVYNLMCDLLNLTPAPNNGTHGSLNHLLKNPVYTPKHPKEVHPLVQCPFTRNPRDNLGCSCNPSILPIEDFQTQFNLTVAEEKIIKHETLPYGRPRVLQKENTICLLSQHQFMSGYSQDILMPLWTSYTVDRNDSFSTEDFSNCLYQDFRIPLSPVHKCSFYKNNTKVSYGFLSPPQLNKNSSGIYSEALLTTNIVPMYQSFQVIWRYFHDTLLRKYAEERNGVNVVSGPVFDFDYDGRCDSLENLRQKRRVIRNQEILIPTHFFIVLTSCKDTSQTPLHCENLDTLAFILPHRTDNSESCVHGKHDSSWVEELLMLHRARITDVEHITGLSFYQQRKEPVSDILKLKTHLPTFSQED